European Patent Application EP 4 458 956 A1, published November 6, 2024. Title: ANTI-MESOTHELIN NANOBODY CHIMERIC ANTIGEN RECEPTOR AND USE THEREOF. Applicant: SHANGHAI CELL THERAPY GROUP CO.,LTD. The sequence listing filed with the application follows.

SEQUENCE LISTING (134 sequences)

SEQ ID NO: 1-3 - skipped (3 entries)

SEQ ID NO: 4 - protein, 8 aa, synthetic construct
  REGION 1..8: note = CDR1
GSIFNINA

SEQ ID NO: 5 - protein, 8 aa, synthetic construct
  REGION 1..8: note = CDR1
GNIFSINA

SEQ ID NO: 6 - protein, 8 aa, synthetic construct
  REGION 1..8: note = CDR1
ESISSIAY

SEQ ID NO: 7 - protein, 8 aa, synthetic construct
  REGION 1..8: note = CDR1
GSSFGLNV

SEQ ID NO: 8 - protein, 8 aa, synthetic construct
  REGION 1..8: note = CDR1
GSVSSINA

SEQ ID NO: 9 - protein, 8 aa, synthetic construct
  REGION 1..8: note = CDR1
GSTFAINA

SEQ ID NO: 10 - protein, 8 aa, synthetic construct
  REGION 1..8: note = CDR1
GSVIDIGA

SEQ ID NO: 11 - protein, 8 aa, synthetic construct
  REGION 1..8: note = CDR1
TPIISIAY

SEQ ID NO: 12 - protein, 8 aa, synthetic construct
  REGION 1..8: note = CDR1
GSIASIDA

SEQ ID NO: 13 - protein, 8 aa, synthetic construct
  REGION 1..8: note = CDR1
GAVSSINA

SEQ ID NO: 14 - protein, 8 aa, synthetic construct
  REGION 1..8: note = CDR1
EHTFTIDA

SEQ ID NO: 15 - protein, 8 aa, synthetic construct
  REGION 1..8: note = CDR1
GSDLSFDA

SEQ ID NO: 16 - protein, 8 aa, synthetic construct
  REGION 1..8: note = CDR1
GDSFGLNV

SEQ ID NO: 17 - protein, 8 aa, synthetic construct
  REGION 1..8: note = CDR1
ANLFTIDA

SEQ ID NO: 18 - protein, 8 aa, synthetic construct
  REGION 1..8: note = CDR1
GDAFSFDA

SEQ ID NO: 19 - protein, 8 aa, synthetic construct
  REGION 1..8: note = CDR1
GSLSSINA

SEQ ID NO: 20 - protein, 8 aa, synthetic construct
  REGION 1..8: note = CDR1
EKTFSIKY

SEQ ID NO: 21 - protein, 8 aa, synthetic construct
  REGION 1..8: note = CDR1
GISFEYYA

SEQ ID NO: 22 - protein, 8 aa, synthetic construct
  REGION 1..8: note = CDR1
GAVSTINA

SEQ ID NO: 23 - protein, 8 aa, synthetic construct
  REGION 1..8: note = CDR1
ASMGSISN

SEQ ID NO: 24 - protein, 8 aa, synthetic construct
  REGION 1..8: note = CDR1
GSHFGLNV

SEQ ID NO: 25 - protein, 8 aa, synthetic construct
  REGION 1..8: note = CDR1
GITLDNYA

SEQ ID NO: 26 - protein, 8 aa, synthetic construct
  REGION 1..8: note = CDR1
GFTFHYYA

SEQ ID NO: 27 - protein, 8 aa, synthetic construct
  REGION 1..8: note = CDR1
GSAFSFDA

SEQ ID NO: 28 - protein, 9 aa, synthetic construct
  REGION 1..9: note = CDR2
ISSSNSDNT

SEQ ID NO: 29 - protein, 9 aa, synthetic construct
  REGION 1..9: note = CDR2
ISSTNSDNT

SEQ ID NO: 30 - protein, 7 aa, synthetic construct
  REGION 1..7: note = CDR2
ISSTGST

SEQ ID NO: 31 - protein, 8 aa, synthetic construct
  REGION 1..8: note = CDR2
IGNGGRTT

SEQ ID NO: 32 - protein, 7 aa, synthetic construct
  REGION 1..7: note = CDR2
MGSGGNT

SEQ ID NO: 33 - protein, 8 aa, synthetic construct
  REGION 1..8: note = CDR2
ISSGGDST

SEQ ID NO: 34 - protein, 7 aa, synthetic construct
  REGION 1..7: note = CDR2
INAGGNT

SEQ ID NO: 35 - protein, 7 aa, synthetic construct
  REGION 1..7: note = CDR2
INSGGKT

SEQ ID NO: 36 - protein, 9 aa, synthetic construct
  REGION 1..9: note = CDR2
ISSSNSDNK

SEQ ID NO: 37 - protein, 7 aa, synthetic construct
  REGION 1..7: note = CDR2
AGRTGTT

SEQ ID NO: 38 - protein, 7 aa, synthetic construct
  REGION 1..7: note = CDR2
TSRDGRI

SEQ ID NO: 39 - protein, 7 aa, synthetic construct
  REGION 1..7: note = CDR2
ISSGGNK

SEQ ID NO: 40 - protein, 7 aa, synthetic construct
  REGION 1..7: note = CDR2
TSRDGRT

SEQ ID NO: 41 - protein, 7 aa, synthetic construct
  REGION 1..7: note = CDR2
MGSDGKT

SEQ ID NO: 42 - protein, 7 aa, synthetic construct
  REGION 1..7: note = CDR2
IDTDGKT

SEQ ID NO: 43 - protein, 12 aa, synthetic construct
  REGION 1..12: note = CDR2
TTSGTTSGGGVT

SEQ ID NO: 44 - protein, 11 aa, synthetic construct
  REGION 1..11: note = CDR2
LVATIGSDGRT

SEQ ID NO: 45 - protein, 8 aa, synthetic construct
  REGION 1..8: note = CDR2
IGNSGRTT

SEQ ID NO: 46 - protein, 7 aa, synthetic construct
  REGION 1..7: note = CDR2
ISSNGNT

SEQ ID NO: 47 - protein, 8 aa, synthetic construct
  REGION 1..8: note = CDR2
ISSSGDST

SEQ ID NO: 48 - protein, 11 aa, synthetic construct
  REGION 1..11: note = CDR3
AAENYDRKDRY

SEQ ID NO: 49 - protein, 11 aa, synthetic construct
  REGION 1..11: note = CDR3
AAENFDRKDRY

SEQ ID NO: 50 - protein, 13 aa, synthetic construct
  REGION 1..13: note = CDR3
AASNKAYNDYDPD

SEQ ID NO: 51 - protein, 10 aa, synthetic construct
  REGION 1..10: note = CDR3
HLRASVTKGY

SEQ ID NO: 52 - protein, 14 aa, synthetic construct
  REGION 1..14: note = CDR3
AADRFGASIHEVDY

SEQ ID NO: 53 - protein, 20 aa, synthetic construct
  REGION 1..20: note = CDR3
NARGCRDFHNPQALCVLRDY

SEQ ID NO: 54 - protein, 14 aa, synthetic construct
  REGION 1..14: note = CDR3
AAEDINYTGTEAYY

SEQ ID NO: 55 - protein, 13 aa, synthetic construct
  REGION 1..13: note = CDR3
AASNKDYNDYDPD

SEQ ID NO: 56 - protein, 11 aa, synthetic construct
  REGION 1..11: note = CDR3
AAEDYDTKDRF

SEQ ID NO: 57 - protein, 14 aa, synthetic construct
  REGION 1..14: note = CDR3
AADKFGADIHEVDY

SEQ ID NO: 58 - protein, 11 aa, synthetic construct
  REGION 1..11: note = CDR3
AVERYSDQSRF

SEQ ID NO: 59 - protein, 10 aa, synthetic construct
  REGION 1..10: note = CDR3
AAGDDPKNYD

SEQ ID NO: 60 - protein, 10 aa, synthetic construct
  REGION 1..10: note = CDR3
HLRVSVTEGY

SEQ ID NO: 61 - protein, 11 aa, synthetic construct
  REGION 1..11: note = CDR3
AAEDYGLGQRS

SEQ ID NO: 62 - protein, 10 aa, synthetic construct
  REGION 1..10: note = CDR3
AAGDDPKDYY

SEQ ID NO: 63 - protein, 14 aa, synthetic construct
  REGION 1..14: note = CDR3
AADRFGAPIHDVDY

SEQ ID NO: 64 - protein, 12 aa, synthetic construct
  REGION 1..12: note = CDR3
AGETGTYPKPEY

SEQ ID NO: 65 - protein, 19 aa, synthetic construct
  REGION 1..19: note = CDR3
AADIHCRGYVLFVPSDFGN

SEQ ID NO: 66 - protein, 14 aa, synthetic construct
  REGION 1..14: note = CDR3
AADKFGADIKEVAY

SEQ ID NO: 67 - protein, 14 aa, synthetic construct
  REGION 1..14: note = CDR3
AADRFGADIREVDY

SEQ ID NO: 68 - protein, 14 aa, synthetic construct
  REGION 1..14: note = CDR3
AVEDRQRPGTENYY

SEQ ID NO: 69 - protein, 10 aa, synthetic construct
  REGION 1..10: note = CDR3
HLRVSVERGY

SEQ ID NO: 70 - protein, 23 aa, synthetic construct
  REGION 1..23: note = CDR3
QVGQFSSSTTPVQAMSVMSLYAD

SEQ ID NO: 71 - protein, 18 aa, synthetic construct
  REGION 1..18: note = CDR3
AGTTRSGYVCYDAEPYDS

SEQ ID NO: 72 - protein, 10 aa, synthetic construct
  REGION 1..10: note = CDR3
AAGDDPKNYS

SEQ ID NO: 73 - protein, 11 aa, synthetic construct
  REGION 1..11: note = CDR1
GFTLRELDEFA

SEQ ID NO: 74 - protein, 8 aa, synthetic construct
  REGION 1..8: note = CDR2
ISGTGGIT

SEQ ID NO: 75 - protein, 16 aa, synthetic construct
  REGION 1..16: note = CDR3
AADERCTDRLIRPPTY

SEQ ID NO: 76 - protein, 121 aa, synthetic construct
  REGION 1..121: note = MSLN VHH
EVQLVESGGGLVQAGGSLRLSCAASGSIFNINAMGWYRQAPGKEWERELVATISSSNSDNTYYKDSVKGRFTISTNTAKNTWYLQMNSLKPEDTAMYYCAAENYDRKDRYWGQGTQVTVSS

SEQ ID NO: 77 - protein, 121 aa, synthetic construct
  REGION 1..121: note = MSLN VHH
QVQLVESGGGLVQAGGSLRLSCTASGNIFSINAMGWYRQPPGKEWERELVATISSTNSDNTYYKESVKGRFTISTNTAKNTWYLQMNSLKPEDTAMYYCAAENFDRKDRYWAQGTQVTVSS

SEQ ID NO: 78 - protein, 119 aa, synthetic construct
  REGION 1..119: note = MSLN VHH
EVQLVESGGGLVQAGGSLRLSCAASESISSIAYMGWYRRISEKERNLVATISSTGSTYYADSVKGRFTISRDNAKNTMYLQMNRLKPEDTAIYYCAASNKAYNDYDPDWGQGTQVTVSS

SEQ ID NO: 79 - protein, 117 aa, synthetic construct
  REGION 1..117: note = MSLN VHH
EVQLVESGGGWVQSGGSLRLACAASGSSFGLNVVGWYRQAPDKQRELVASIGNGGRTTDYADSVKGRFTISSDNAKNTVFLQMNDLKPEDTAVYYCHLRASVTKGYWGQGTQVTVSS

SEQ ID NO: 80 - protein, 120 aa, synthetic construct
  REGION 1..120: note = MSLN VHH
QVQLVESGGGLVQAGGSLRLSCAASGSVSSINAMGWYRQGTGEVRKLVATMGSGGNTYYADSVKGRFFITRDYSKNTVSLQMNNLTPEDSATYYCAADRFGASIHEVDYWGKGTLVTVSS

SEQ ID NO: 81 - protein, 127 aa, synthetic construct
  REGION 1..127: note = MSLN VHH
QVQLVESGGDLVQTGGSLRLSCVVSGSTFAINAMGWYRQAPGKERELVAAISSGGDSTHYADDVKGRFTISRDNAENTMYLQMKSLKPEDTAVYVCNARGCRDFHNPQALCVLRDYWGQGTQVTVSS

SEQ ID NO: 82 - protein, 120 aa, synthetic construct
  REGION 1..120: note = MSLN VHH
EVQLVESGGGSVQAGGSLKISCAASGSVIDIGAMGWYRHITEKERKLVATINAGGNTYYADSVKGRFTISRDNAKYTVYLQMNSLKPEDTAMYYCAAEDINYTGTEAYYWGQGTQVTVSS

SEQ ID NO: 83 - protein, 119 aa, synthetic construct
  REGION 1..119: note = MSLN VHH
QVQVVESGGGFVQAGGSLRLSCAASTPIISIAYMGWYRQISEKERQLVATINSGGKTYYADSVKGRFTISRDNAKNTLYLQMNMLKPEDTGMYYCAASNKDYNDYDPDWGQGTQVTVSS

SEQ ID NO: 84 - protein, 121 aa, synthetic construct
  REGION 1..121: note = MSLN VHH
QVQLVETGGGSVQAGGSLRLSCAASGSIASIDAMGWYRQVPGKEWERELVATISSSNSDNKYYKDSVKGRFTISTNIAKNTWYLQMNNLKPEDTAMYYCAAEDYDTKDRFWGQGTQVTVSS

SEQ ID NO: 85 - protein, 120 aa, synthetic construct
  REGION 1..120: note = MSLN VHH
EVQLQESGGGLVQAGGSLRLSCAASGAVSSINAMGWYRQTPEKVRKLVATMGSGGNTYYADSVKGRFTISRDYAKNTVALQMNNLIPEDTAVYYCAADKFGADIHEVDYWGKGTLVTVSS

SEQ ID NO: 86 - protein, 119 aa, synthetic construct
  REGION 1..119: note = MSLN VHH
EVQLVESGGGLVQAGGSLTLSCAASEHTFTIDAMGYYRQIPGRRNERQLVAAAGRTGTTYYNDAVKDRFTIYRDTSKETIILQMNNLRPEDTTMYYCAVERYSDQSRFFGPGTQVTVSS

SEQ ID NO: 87 - protein, 118 aa, synthetic construct
  REGION 1..118: note = MSLN VHH
EVQLVESGGGLVQPGGSLRLSCVASGSDLSFDAMGWYRQFSATVRERQLVVATSRDGRIYYGDSVKGRFTASRDNLKNSVDLEMNNLKPEDTAIYYCAAGDDPKNYDWGPGTQVTVSS

SEQ ID NO: 88 - protein, 117 aa, synthetic construct
  REGION 1..117: note = MSLN VHH
EVQLVESGGGWVQSGGSLRLACAASGDSFGLNVVGWYRLAPDKQRELVASIGNGGRTTDYADSVKGRFTISSDNAKNTVFLQMNDLKPEDTAMYYCHLRVSVTEGYWGQGTQVTVSS

SEQ ID NO: 89 - protein, 117 aa, synthetic construct
  REGION 1..117: note = MSLN VHH
QVQLVESGGGSAQAGGSLILSCVASANLFTIDALGWYRQAPGPKRELVAAISSGGNKYYADAVKGRFTISRDTLTKTMWLQMNNLKPEDTAMYYCAAEDYGLGQRSWGMGTQVTVSS

SEQ ID NO: 90 - protein, 118 aa, synthetic construct
  REGION 1..118: note = MSLN VHH
QVQLVESGGGLVQAGGSLSLSCVASGDAFSFDAMGWYRQFSGKVNERQLVVATSRDGRTAYGERVKGRFTASRDNSKNTLSLVMNNLQVEDTAIYYCAAGDDPKDYYWGQGTQVTVSS

SEQ ID NO: 91 - protein, 119 aa, synthetic construct
  REGION 1..119: note = MSLN VHH
QVQLVESGGGLVQAGGSLSLSCAASGSLSSINAMGWYRQLPEMRQLVATMGSDGKTYYADSVKGRFTISRDYAKYTVSLQMNNLRPEDTAIYYCAADRFGAPIHDVDYWGKGTLVTVSV

SEQ ID NO: 92 - protein, 118 aa, synthetic construct
  REGION 1..118: note = MSLN VHH
EVQLVESGGGLVQAGGSLRLSCSASEKTFSIKYMGYYRQGPGIERKLVATIDTDGKTWYADSVKGRFTISRENGENEIGLEMNRLKPEDTAMYYCAGETGTYPKPEYWGQGTQVTVSS

SEQ ID NO: 93 - protein, 130 aa, synthetic construct
  REGION 1..130: note = MSLN VHH
QVQLVESGGGLVQAGGSLRLSCAVSGISFEYYAIGWFRQAPGKEREAVSCTTSGTTSGGGVTDYADSLKGRFTISRDVAKNTVYLQMNNLTPEDTAVYYCAADIHCRGYVLFVPSDFGNWGQGTQVTVSS

SEQ ID NO: 94 - protein, 119 aa, synthetic construct
  REGION 1..119: note = MSLN VHH
EVQLVESGGGTVQPGESLRLSCEASGAVSTINAMGWYRQTPEMRKLVATMGSGGNTYYADSVKGRFTISRDFAGNTVDLQMNDLKPEDTGVYFCAADKFGADIKEVAYWGKGTLVTVSS

SEQ ID NO: 95 - protein, 120 aa, synthetic construct
  REGION 1..120: note = MSLN VHH
QVQLVESGGGSVQAGGSLTLSCAASGAVSSINAMGWYRQTPEKVRQLVATMGSGGNTYYAASVKGRFTISRDYAKNTVALQMNHLLPEDTAVYYCAADRFGADIREVDYWGKGTQVTVSS

SEQ ID NO: 96 - protein, 124 aa, synthetic construct
  REGION 1..124: note = MSLN VHH
QVQLVESGGGLVQAGGSLRLSCAASASMGSISNMGWYRQAPGKERGNERNLVATIGSDGRTYYADSVKGRFTISRDNVKNTMILQMNFLKPEDTAMYYCAVEDRQRPGTENYYWGQGTQVTVSS

SEQ ID NO: 97 - protein, 117 aa, synthetic construct
  REGION 1..117: note = MSLN VHH
EVQLVESGGGLVQAGGSLRLSCAASGSHFGLNVVGWYRQAPGKQRELVASIGNSGRTTDYADSVKGRFTISKDNAQNTIYLQMNNLKPEDTAMYRCHLRVSVERGYWGQGTQVTVSS

SEQ ID NO: 98 - protein, 129 aa, synthetic construct
  REGION 1..129: note = MSLN VHH
QVQLVESGGGLVQPGGSLRLSCAASGITLDNYAIAWFRQAPGKKREGVSCISSNGNTYYQPSVKGRFTIARDNAKNTVYLHMNNLNPEDTAVYYCQVGQFSSSTTPVQAMSVMSLYADWGQGTQVTVSS

SEQ ID NO: 99 - protein, 125 aa, synthetic construct
  REGION 1..125: note = MSLN VHH
QVQLVESGGGLVQPGGSLRLSCAASGFTFHYYAIGWFRQAPGKEREGVSCISSSGDSTWFSDSVKGRFTVSRDNAKNIVHLQMNNLKPEDTAVYYCAGTTRSGYVCYDAEPYDSWGQGTQVTVSS

SEQ ID NO: 100 - protein, 118 aa, synthetic construct
  REGION 1..118: note = MSLN VHH
QVQLVESGGGLVQSGGSLRLSCVASGSAFSFDAMGWYRQFSATRRERQLVVATSRDGRTYYADSVKGRFTATRDNSKNSLYLEMNSLKPEDTAIYYCAAGDDPKNYSWGQGTQVTVSS

SEQ ID NO: 101 - protein, 126 aa, synthetic construct
  REGION 1..126: note = MSLN VHH
QLQLGASGGGLVQPGGSLRLSCALSGFTLRELDEFAIGWFRQAPGKEREGVSCISGTGGITHYADSVKGRFTISRDIAKTTVYLQMNSLNSEDTAVYYCAADERCTDRLIRPPTYWGQGTQVTVSS

SEQ ID NO: 102 - protein, 126 aa, synthetic construct
  REGION 1..126: note = MSLN VHH
EVQLVASGGGLVQPGGSLRLSCALSGFTLRELDEFAIGWFRQAPGKEREGVSCISGTGGITHYADSVKGRFTISRDNSKTTVYLQMNSLRAEDTAVYYCAADERCTDRLIRPPTYWGQGTQVTVSS

SEQ ID NO: 103 - protein, 126 aa, synthetic construct
  REGION 1..126: note = MSLN VHH
QVQLVASGGGLVQPGGSLRLSCALSGFTLRELDEFAIGWFRQAPGKEREGVSCISGTGGITHYADSVKGRFTISRDNSKTTVYLQMNSLRAEDTAVYYCAADERCTDRLIRPPTYWGQGTQVTVSS

SEQ ID NO: 104 - protein, 126 aa, synthetic construct
  REGION 1..126: note = MSLN VHH
ELQLVASGGGLVQPGGSLRLSCALSGFTLRELDEFAIGWFRQAPGKEREGVSCISGTGGITHYADSVKGRFTISRDNSKTTVYLQMNSLRAEDTAVYYCAADERCTDRLIRPPTYWGQGTQVTVSS

SEQ ID NO: 105 - protein, 126 aa, synthetic construct
  REGION 1..126: note = MSLN VHH
EVQLGASGGGLVQPGGSLRLSCALSGFTLRELDEFAIGWFRQAPGKEREGVSCISGTGGITHYADSVKGRFTISRDNSKTTVYLQMNSLRAEDTAVYYCAADERCTDRLIRPPTYWGQGTQVTVSS

SEQ ID NO: 106 - protein, 126 aa, synthetic construct
  REGION 1..126: note = MSLN VHH
EVQLVASGGGLVQPGGSLRLSCALSGFTLRELDEFAIGWFRQAPGKEREGVSCISGTGGITHYADSVKGRFTISRDNSKTTVYLQMNSLNAEDTAVYYCAADERCTDRLIRPPTYWGQGTQVTVSS

SEQ ID NO: 107 - protein, 126 aa, synthetic construct
  REGION 1..126: note = MSLN VHH
EVQLVASGGGLVQPGGSLRLSCALSGFTLRELDEFAIGWFRQAPGKEREGVSCISGTGGITHYADSVKGRFTISRDNSKTTVYLQMNSLRSEDTAVYYCAADERCTDRLIRPPTYWGQGTQVTVSS

SEQ ID NO: 108 - protein, 126 aa, synthetic construct
  REGION 1..126: note = MSLN VHH
ELQLGASGGGLVQPGGSLRLSCALSGFTLRELDEFAIGWFRQAPGKEREGVSCISGTGGITHYADSVKGRFTISRDNSKTTVYLQMNSLRAEDTAVYYCAADERCTDRLIRPPTYWGQGTQVTVSS

SEQ ID NO: 109 - protein, 126 aa, synthetic construct
  REGION 1..126: note = MSLN VHH
QLQLGESGGGLVQPGGSLRLSCALSGFTLRELDEFAIGWFRQAPGKEREGVSCISGTGGITHYADSVKGRFTISRDIAKTTVYLQMNSLNSEDTAVYYCAADERCTDRLIRPPTYWGQGTQVTVSS

SEQ ID NO: 110 - protein, 126 aa, synthetic construct
  REGION 1..126: note = MSLN VHH
QLQLVASGGGLVQPGGSLRLSCALSGFTLRELDEFAIGWFRQAPGKEREGVSCISGTGGITHYADSVKGRFTISRDIAKTTVYLQMNSLNSEDTAVYYCAADERCTDRLIRPPTYWGQGTQVTVSS

SEQ ID NO: 111 - protein, 126 aa, synthetic construct
  REGION 1..126: note = MSLN VHH
QLQLVESGGGLVQPGGSLRLSCALSGFTLRELDEFAIGWFRQAPGKEREGVSCISGTGGITHYADSVKGRFTISRDIAKTTVYLQMNSLNSEDTAVYYCAADERCTDRLIRPPTYWGQGTQVTVSS

SEQ ID NO: 112 - protein, 126 aa, synthetic construct
  REGION 1..126: note = MSLN VHH
QLQLGASGGGLVQPGGSLRLSCAASGFTLRELDEFAIGWFRQAPGKEREGVSCISGTGGITHYADSVKGRFTISRDIAKTTVYLQMNSLNSEDTAVYYCAADERCTDRLIRPPTYWGQGTQVTVSS

SEQ ID NO: 113 - protein, 126 aa, synthetic construct
  REGION 1..126: note = MSLN VHH
EVQLGASGGGLVQPGGSLRLSCALSGFTLRELDEFAIGWFRQAPGKEREGVSCISGTGGITHYADSVKGRFTISRDIAKTTVYLQMNSLNSEDTAVYYCAADERCTDRLIRPPTYWGQGTQVTVSS

SEQ ID NO: 114 - protein, 126 aa, synthetic construct
  REGION 1..126: note = MSLN VHH
QLQLGASGGGLVQPGGSLRLSCALSGFTLRELDEFAIGWFRQAPGKEREGVSCISGTGGITHYADSVKGRFTISRDNSKTTVYLQMNSLNSEDTAVYYCAADERCTDRLIRPPTYWGQGTQVTVSS

SEQ ID NO: 115 - protein, 126 aa, synthetic construct
  REGION 1..126: note = MSLN VHH
QLQLGASGGGLVQPGGSLRLSCALSGFTLRELDEFAIGWFRQAPGKEREGVSCISGTGGITHYADSVKGRFTISRDIAKNTVYLQMNSLNSEDTAVYYCAADERCTDRLIRPPTYWGQGTQVTVSS

SEQ ID NO: 116 - protein, 126 aa, synthetic construct
  REGION 1..126: note = MSLN VHH
QLQLGASGGGLVQPGGSLRLSCALSGFTLRELDEFAIGWFRQAPGKEREGVSCISGTGGITHYADSVKGRFTISRDIAKTTLYLQMNSLNSEDTAVYYCAADERCTDRLIRPPTYWGQGTQVTVSS

SEQ ID NO: 117 - protein, 126 aa, synthetic construct
  REGION 1..126: note = MSLN VHH
QLQLGASGGGLVQPGGSLRLSCALSGFTLRELDEFAIGWFRQAPGKEREGVSCISGTGGITHYADSVKGRFTISRDIAKTTVYLQMNSLRAEDTAVYYCAADERCTDRLIRPPTYWGQGTQVTVSS

SEQ ID NO: 118 - protein, 126 aa, synthetic construct
  REGION 1..126: note = MSLN VHH
ELQLGASGGGLVQPGGSLRLSCALSGFTLRELDEFAIGWFRQAPGKEREGVSCISGTGGITHYADSVKGRFTISRDNSKNTLYLQMNSLRAEDTAVYYCAADERCTDRLIRPPTYWGQGTQVTVSS

SEQ ID NO: 119 - protein, 126 aa, synthetic construct; identical to SEQ ID NO: 115
  REGION 1..126: note = MSLN VHH

SEQ ID NO: 120 - protein, 126 aa, synthetic construct; identical to SEQ ID NO: 116
  REGION 1..126: note = MSLN VHH

SEQ ID NO: 121 - protein, 384 aa, synthetic construct
  REGION 1..384: note = CAR
MALPVTALLLPLALLLHAARPSQVQLVASGGGLVQPGGSLRLSCALSGFTLRELDEFAIGWFRQAPGKEREGVSCISGTGGITHYADSVKGRFTISRDNSKTTVYLQMNSLRAEDTAVYYCAADERCTDRLIRPPTYWGQGTQVTVSSFVPVFLPAKPTTTPAPRPPTPAPTIASQPLSLRPEACRPAAGGAVHTRGLDFACDPFWVLVVVGGVLACYSLLVTVAFIIFWVRSKRSRLLHSDYMNMTPRRPGPTRKHYQPYAPPRDFAAYRSRVKFSRSADAPAYQQGQNQLYNELNLGRREEYDVLDKRRGRDPEMGGKPRRKNPQEGLYNELQKDKMAEAYSEIGMKGERRRGKGHDGLYQGLSTATKDTYDALHMQALPPR

SEQ ID NO: 122 - protein, 377 aa, synthetic construct
  REGION 1..377: note = CAR
MALPVTALLLPLALLLHAARPSQVQVVESGGGFVQAGGSLRLSCAASTPIISIAYMGWYRQISEKERQLVATINSGGKTYYADSVKGRFTISRDNAKNTLYLQMNMLKPEDTGMYYCAASNKDYNDYDPDWGQGTQVTVSSFVPVFLPAKPTTTPAPRPPTPAPTIASQPLSLRPEACRPAAGGAVHTRGLDFACDPFWVLVVVGGVLACYSLLVTVAFIIFWVRSKRSRLLHSDYMNMTPRRPGPTRKHYQPYAPPRDFAAYRSRVKFSRSADAPAYQQGQNQLYNELNLGRREEYDVLDKRRGRDPEMGGKPRRKNPQEGLYNELQKDKMAEAYSEIGMKGERRRGKGHDGLYQGLSTATKDTYDALHMQALPPR

SEQ ID NO: 123 - protein, 378 aa, synthetic construct
  REGION 1..378: note = CAR
MALPVTALLLPLALLLHAARPSEVQLQESGGGLVQAGGSLRLSCAASGAVSSINAMGWYRQTPEKVRKLVATMGSGGNTYYADSVKGRFTISRDYAKNTVALQMNNLIPEDTAVYYCAADKFGADIHEVDYWGKGTLVTVSSFVPVFLPAKPTTTPAPRPPTPAPTIASQPLSLRPEACRPAAGGAVHTRGLDFACDPFWVLVVVGGVLACYSLLVTVAFIIFWVRSKRSRLLHSDYMNMTPRRPGPTRKHYQPYAPPRDFAAYRSRVKFSRSADAPAYQQGQNQLYNELNLGRREEYDVLDKRRGRDPEMGGKPRRKNPQEGLYNELQKDKMAEAYSEIGMKGERRRGKGHDGLYQGLSTATKDTYDALHMQALPPR

SEQ ID NO: 124 - protein, 8 aa, synthetic construct
  REGION 1..8: note = PD1 CDR1
GDTSFISA

SEQ ID NO: 125 - protein, 7 aa, synthetic construct
  REGION 1..7: note = PD1 CDR2
ITNTGIT

SEQ ID NO: 126 - protein, 17 aa, synthetic construct
  REGION 1..17: note = PD1 CDR3
NAGAPPPGGLGYDESDY

SEQ ID NO: 127 - protein, 123 aa, synthetic construct
  REGION 1..123: note = PD1 VHH
QVQLVESGGGLVQAGGSLRLSCAASGDTSFISAAGWYRQAPGKERELVAAITNTGITYYPDSVKGRFTISRDNAKNTVYLQMNNLKPEDTAVYYCNAGAPPPGGLGYDESDYWGQGTQVTVSS

SEQ ID NO: 128 - protein, 8 aa, synthetic construct
  REGION 1..8: note = PD1 CDR1
GRPFSIYD

SEQ ID NO: 129 - protein, 8 aa, synthetic construct
  REGION 1..8: note = PD1 CDR2
INLARGNT

SEQ ID NO: 130 - protein, 17 aa, synthetic construct
  REGION 1..17: note = PD1 CDR3
GVDRRQYGLGIPPLADH

SEQ ID NO: 131 - protein, 124 aa, synthetic construct
  REGION 1..124: note = PD1 VHH
EVQLVESGGGLVQPGGSLRLSCAASGRPFSIYDMGWFRQAPDKERESVAVINLARGNTYYADSVKGRFTISRDNAKNTVYLQMNSLRAEDTAVYSCGVDRRQYGLGIPPLADHWGQGTQVTVSS

SEQ ID NO: 132 - protein, 229 aa, synthetic construct
  REGION 1..229: note = MSLN CH
ESKYGPPCPPCPAPEFLGGPSVFLFPPKPKDTLMISRTPEVTCVVVDVSQEDPEVQFNWYVDGVEVHNAKTKPREEQFNSTYRVVSVLTVLHQDWLNGKEYKCKVSNKGLPSSIEKTISKAKGQPREPQVYTLPPSQEEMTKNQVSLTCLVKGFYPSDIAVEWESNGQPENNYKTTPPVLDSDGSFFLYSRLTVDKSRWQEGNVFSCSVMHEALHNHYTQKSLSLSLGK

SEQ ID NO: 133 - protein, 217 aa, synthetic construct
  REGION 1..217: note = PD1 Fc
APEFLGGPSVFLFPPKPKDTLMISRTPEVTCVVVDVSQEDPEVQFNWYVDGVEVHNAKTKPREEQFNSTYRVVSVLTVLHQDWLNGKEYKCKVSNKGLPSSIEKTISKAKGQPREPQVYTLPPSQEEMTKNQVSLTCLVKGFYPSDIAVEWESNGQPENNYKTTPPVLDSDGSFFLYSRLTVDKSRWQEGNVFSCSVMHEALHNHYTQKSLSLSLGK

SEQ ID NO: 134 - protein, 143 aa, synthetic construct
  REGION 1..143: note = antibody for PD1 nanobody
MEAPAQLLFLLLLWLPDTTGEVQLVESGGGLVQPGGSLRLSCSASGDTSFISAAGWYRQAPGKERELVSAITNTGITYYPDSVKGRFTISRDNSKNTVYLQMNSLRAEDTAVYYCNAGAPPPGGLGYDESDYWGQGTQVTVSS